European Patent Application EP 4 252 780 A1, published October 4, 2023. Title: Oral formulation of physiological active material conjugate linked with biotin moiety, fatty acid moiety or a combination thereof. Applicant: D&D Pharmatech. The sequence listing filed with the application follows.

SEQUENCE LISTING (42 sequences)

SEQ ID NO: 1 - protein, 29 aa, Artificial Sequence
  Glucagon derivative
  VARIANT (2): Xaa is 2-Aminoisobutyric acid
HXQGTFTSDYSKYLDEQAAKEFVQWLMNT

SEQ ID NO: 2 - protein, 30 aa, Artificial Sequence
  GLP-1
HAEGTFTSDVSSYLEGQAAKEFIAWLVKGR

SEQ ID NO: 3 - protein, 33 aa, Artificial Sequence
  GLP-2
HADGSFSDEMNTILDNLAARDFINWLIQTKITD

SEQ ID NO: 4 - protein, 42 aa, Artificial Sequence
  GIP
YAEGTFISDYSIAMDKIHQQDFVNWLLAQKGKKNDWKHNITQ

SEQ ID NO: 5 - protein, 39 aa, Artificial Sequence
  EXENDIN-4
HGEGTFTSDLSKQMEEEAVRLFIEWLKNGGPSSGAPPPS

SEQ ID NO: 6 - protein, 34 aa, Artificial Sequence
  PTH
SVSEIQLMHNLGKHLNSMERVEWLRKKLQDVHNF

SEQ ID NO: 7 - protein, 29 aa, Artificial Sequence
  Glucagon
HSQGTFTSDYSKYLDSRRAQDFVQWLMNT

SEQ ID NO: 8 - protein, 30 aa, Artificial Sequence
  Glucagon derivative
  VARIANT (2): X is 2-Aminoisobutyric acid
HXQGTFTSDYSKYLDEQAAKEFVQWLMNTC

SEQ ID NO: 9 - protein, 31 aa, Artificial Sequence
  GLP-1 derivative
HAEGTFTSDVSSYLEGQAAKEFIAWLVKGRC

SEQ ID NO: 10 - protein, 34 aa, Artificial Sequence
  GLP-2 derivative
HADGSFSDEMNTILDNLAARDFINWLIQTKITDC

SEQ ID NO: 11 - protein, 43 aa, Artificial Sequence
  GIP derivative
YAEGTFISDYSIAMDKIHQQDFVNWLLAQKGKKNDWKHNITQC

SEQ ID NO: 12 - protein, 40 aa, Artificial Sequence
  EXENDIN-4 derivative
HGEGTFTSDLSKQMEEEAVRLFIEWLKNGGPSSGAPPPSC

SEQ ID NO: 13 - protein, 35 aa, Artificial Sequence
  PTH derivative
SVSEIQLMHNLGKHLNSMERVEWLRKKLQDVHNFC

SEQ ID NO: 14 - protein, 30 aa, Artificial Sequence
  Glucagon derivative
HSQGTFTSDYSKYLDSRRAQDFVQWLMNTC

SEQ ID NO: 15 - protein, 21 aa, Artificial Sequence
  Insulin chain A derivative
GIVEQCCTSICSLEQLENYCN

SEQ ID NO: 16 - protein, 30 aa, Artificial Sequence
  Insulin chain B
FVNQHLCGSHLVEALYLVCGERGFFYTPKT

SEQ ID NO: 17 - protein, 21 aa, Artificial Sequence
  Insulin chain A
GIVEQCCTSICSLYQLENYCN

SEQ ID NO: 18 - protein, 40 aa, Artificial Sequence
  Exendin-4 derivative
HGEGTFTSDLSKQMEEEAVRLFIEWLKNGGPSSGAPPPSK

SEQ ID NO: 19 - protein, 42 aa, Artificial Sequence
  Exendin-4 derivative
HGEGTFTSDLSKQMEEEAVRLFIEWLKNGGPSSGAPPPSKKK

SEQ ID NO: 20 - protein, 40 aa, Artificial Sequence
  Exendin-4 derivative
  VARIANT (2): X is 2-Aminoisobutyric acid
HXEGTFTSDLSKQMEEEAVRLFIEWLKNGGPSSGAPPPSK

SEQ ID NO: 21 - protein, 42 aa, Artificial Sequence
  Exendin-4 derivative
  VARIANT (2): X is 2-Aminoisobutyric acid
HXEGTFTSDLSKQMEEEAVRLFIEWLKNGGPSSGAPPPSKKK

SEQ ID NO: 22 - protein, 37 aa, Artificial Sequence [sequence omitted]

SEQ ID NO: 23 - protein, 38 aa, Artificial Sequence
  Amylin derivative
KCNTATCATQRLANFLVHSSNNFGAILSSTNVGSNTYK

SEQ ID NO: 24 - protein, 37 aa, Artificial Sequence
  Amylin derivative
KCNTATCATQRLANFLVHSSNNFGPILPPTNVGSNTY

SEQ ID NO: 25 - protein, 38 aa, Artificial Sequence
  Amylin derivative
KCNTATCATQRLANFLVHSSNNFGPILPPTNVGSNTYK

SEQ ID NO: 26 - protein, 37 aa, Artificial Sequence
  Amylin derivative
KCNTATCATQRLADFLRHSSPNFGAIPSSTNVGSRTY

SEQ ID NO: 27 - protein, 38 aa, Artificial Sequence
  Amylin derivative
KCNTATCATQRLADFLRHSSPNFGAIPSSTNVGSRTYK

SEQ ID NO: 28 - protein, 37 aa, Artificial Sequence
  Amylin derivative
KCNTATCATQRLADFLRHSSNNFGAIPSSTNVGSRTY

SEQ ID NO: 29 - protein, 38 aa, Artificial Sequence
  Amylin derivative
KCNTATCATQRLADFLRHSSNNFGAIPSSTNVGSRTYK

SEQ ID NO: 30 - protein, 37 aa, Artificial Sequence
  Amylin derivative
RCNTATCATQRLADFLRHSSNNFGAIPSSTNVGSKTY

SEQ ID NO: 31 - protein, 38 aa, Artificial Sequence
  Amylin derivative
RCNTATCATQRLADFLRHSSNNFGAIPSSTNVGSKTYK

SEQ ID NO: 32 - protein, 39 aa, Artificial Sequence
  Exendin-4 derivative
  VARIANT (2): X is 2-Aminoisobutyric acid
HXQGTFTSDKSKYLDERAAQDFVQWLLDGGPSSGAPPPS

SEQ ID NO: 33 - protein, 39 aa, Artificial Sequence
  Exendin-4 derivative
  VARIANT (2): X is 2-Aminoisobutyric acid
HXQGTFTSDKSKYLDERAAQDFVQWLMDGGPSSGAPPPS

SEQ ID NO: 34 - protein, 39 aa, Artificial Sequence
  Exendin-4 derivative
  VARIANT (2): X is 2-Aminoisobutyric acid
HXQGTFTSDKSKYLDKIAAQDFVQWLIDGGPSSGAPPPS

SEQ ID NO: 35 - protein, 39 aa, Artificial Sequence
  Exendin-4 derivative
  VARIANT (2): X is 2-Aminoisobutyric acid
HXQGTFTSDKSWYLDKIAAQDFVQWLLGGGPSSGAPPPS

SEQ ID NO: 36 - protein, 39 aa, Artificial Sequence
  Exendin-4 derivative
  VARIANT (2): X is 2-Aminoisobutyric acid
HXQGTFTSDKSWYLDERAAQDFVQWLMGGGPSSGAPPPS

SEQ ID NO: 37 - protein, 39 aa, Artificial Sequence
  Exendin-4 derivative
  VARIANT (2): X is 2-Aminoisobutyric acid
HXQGTFTSDKSKWLDKIAAQDFVQWLIGGGPSSGAPPPS

SEQ ID NO: 38 - protein, 40 aa, Artificial Sequence
  Exendin-4 derivative
  VARIANT (2): X is 2-Aminoisobutyric acid
HXEGTFTSDLSKQMEEEAVRLFIEWLKNGGPSSGAPPPSC

SEQ ID NO: 39 - protein, 40 aa, Artificial Sequence; identical to SEQ ID NO: 38
  Exendin-4 derivative
  VARIANT (2): X is 2-Aminoisobutyric acid
  VARIANT (1): H1 is Des-amino-His

SEQ ID NO: 40 - protein, 30 aa, Artificial Sequence
  Glucagon derivative
  VARIANT (2): X is 2-Aminoisobutyric acid
HXQGTFTSDYSKYLDEQAAKEFVQWLMNTK

SEQ ID NO: 41 - protein, 30 aa, Artificial Sequence
  Glucagon derivative
  VARIANT (2): X is 2-Aminoisobutyric acid
HXQGTFTSDYSKYLDEKRAKEFVQWLMNTC

SEQ ID NO: 42 - protein, 192 aa, Artificial Sequence
  Human growth hormone derivative
MFPTIPLSRLFDNAMLRAHRLHQLAFDTYQEFEEAYIPKEQKISFLQNPQTSLCFSESIPTPSNREETQQKSNLELLRISLLLIQSWLEPVQFLRSVFANSLVYGASDSNVYDLLKDLEEGIQTLMGRLEDGSPRTGQIFKQTYSKFDTNSHNDDALLKNYGLLYCFRKDMDKVETFLRIVQCRSVEGSCGF